European Patent Application EP 4 311 430 A1, published January 31, 2024. Title: CHLOROTOLURON TOLERANCE GENE AND METHODS OF USE THEREOF. Applicant: LIMAGRAIN EUROPE. Application EP. The sequence listing filed with the application follows.

SEQUENCE LISTING (14 sequences)

SEQ ID NO: 1 - protein, 531 aa, Triticum aestivum
MAAQTVLPLLLSPQALLLYLLLIPLVILLRATSTRPAGERAAADNHGGRPLPSPPNKLPLIGHLHLVGPDPHVSLAILAAKHGDGGLMLLRLGQTRALVVSSPRAAEAVLRTQDHVFASRPPNALVDALLDGGADVAFAPYGEFWRQARRLVTTHLLSARKLHSLRRGREGEARLVMAKIQGAAAAGAPVDMTRLLGSFTNDIACRAVSGKFFREEGRNELFREAIDGNVAAFGGFSLLDYFPGLAKVGVLTRVVFAKNSQLKRKWDELLDKIIDDHVSKASAQEQHHKHDQQEDQETDFVDVLLSLQEEYSLTRQHIKAILMDMFVAGTDTSYIVLECAMAELMRKPNLMAKLQAEVREKTPKGQQMVTEDDLASMAYLKATVKETLRLHPPLPLLLPHLSMTECDIDGYKVPARTRVIVNAWALGRDPGSWEAADKFMPERFVDVVSPDFKGRDFQFLPFGAGRRICPGINFGMASVEIMLANLVYCYDWELPDGMRQEDLDMTDVFGMTMRRKEKLFLVPRTRDVNHA

SEQ ID NO: 2 - DNA, 1596 bp, Triticum aestivum
  source 1..1596: mol_type = other DNA
atggcggctcaaacagtgctaccactgctcttatctccccaagcactattgctctatctcttgctcatccctctggtgatcctcctccgggcaacaagcacgagaccggccggcgagcgagccgcagcggacaaccatgggggccgtcccctcccttcgcctccgaacaagctccctctcatcggccacctgcacctggtcggccccgacccgcacgtctccctcgccatcctcgccgccaagcacggcgacggcggcctcatgctcctccgcctcggccagacgcgcgccctcgtcgtctcctccccgcgcgccgccgaggcggtcctgcgcacgcaggaccacgtcttcgcctcgcggcctccgaacgcgctcgtcgacgccctcctggacggcggcgccgacgtcgccttcgccccctacggcgagttctggcggcaggccaggaggctggtcaccacgcacctgctcagcgccaggaagctgcactcgctccgccgcggccgcgagggggaggcgcgcctggtgatggccaagatccagggcgcggcggccgccggcgcccccgtggacatgacgaggctgctcggcagcttcaccaacgacatagcgtgccgcgccgtgtccgggaagttcttccgggaggaaggccggaacgagctgttcagggaggcgatcgacgggaacgtggccgcgtttggcgggttcagcctgctggactacttcccgggcctggccaaggtgggcgtgctcacgcgagtggttttcgccaagaacagtcagttgaagaggaaatgggacgagctgctcgacaagatcatcgacgaccatgtcagcaaagcatcggcacaggagcaacaccacaagcacgatcagcaagaagatcaagagacagacttcgtcgatgtgctcctcagtcttcaggaggagtacagtctcaccagacagcatatcaaggccatactgatggacatgtttgtggcaggcacagatacgtcatacatagttcttgagtgcgccatggctgagctcatgcgaaagccgaacctcatggccaaacttcaagctgaggtgagggaaaagacacccaagggccaacaaatggtgaccgaggacgacttggccagcatggcctacctaaaggccaccgtgaaggaaacgctccggctacacccaccgctgccgctcctcctcccgcacctctccatgaccgaatgcgacatcgacggctataaagtccccgccagaacccgtgtcatcgtaaacgcttgggctcttggtagagaccctggatcgtgggaggctgccgacaagttcatgccggagaggtttgtggacgtcgtgtcccccgacttcaaagggagggattttcagtttctgccgtttggagctggccgaaggatatgtcccgggataaattttgggatggcgtctgtggagatcatgcttgccaaccttgtctattgttatgattgggagctcccggacggcatgcggcaagaggacctggatatgactgatgtgtttggcatgacgatgcgtcggaaggagaagttatttcttgtcccgagaacacgagatgttaatcatgcataa

SEQ ID NO: 3 - DNA, 2999 bp, Triticum aestivum
  source 1..2999: mol_type = genomic DNA
ctatatcacttggcttagacttggttaagtctcagttgactgagatctagctacatccttatattaaagatccaacggctgctctactttctccttccacgaaattaacttacccaaattgtaaatttagtcaacttacatgtaactattgcagaaggaaggaaaaacatatttcccatgcattggcaggtggataagatacgtacatatgtgatcatggttgcgccgcgcatgtccatcgatggagaaattcaagtccaccaccactaaacgatgaacagaagtggagaaggacacgcaccaaactccaaagtccaaacctcattgtcacgtagcaaatcgcgagcatgggctacgcatccagtcgtggtcagaagatcacagtgatcactcttgtcgaccagctacaaatacgacaccaagggagggtgctacaagcaggccatggcggctcaaacagtgctaccactgctcttatctccccaagcactattgctctatctcttgctcatccctctggtgatcctcctccgggcaacaagcacgagaccggccggcgagcgagccgcagcggacaaccatgggggccgtcccctcccttcgcctccgaacaagctccctctcatcggccacctgcacctggtcggccccgacccgcacgtctccctcgccatcctcgccgccaagcacggcgacggcggcctcatgctcctccgcctcggccagacgcgcgccctcgtcgtctcctccccgcgcgccgccgaggcggtcctgcgcacgcaggaccacgtcttcgcctcgcggcctccgaacgcgctcgtcgacgccctcctggacggcggcgccgacgtcgccttcgccccctacggcgagttctggcggcaggccaggaggctggtcaccacgcacctgctcagcgccaggaagctgcactcgctccgccgcggccgcgagggggaggcgcgcctggtgatggccaagatccagggcgcggcggccgccggcgcccccgtggacatgacgaggctgctcggcagcttcaccaacgacatagcgtgccgcgccgtgtccgggaagttcttccgggaggaaggccggaacgagctgttcagggaggcgatcgacgggaacgtggccgcgtttggcgggttcagcctgctggactacttcccgggcctggccaaggtgggcgtgctcacgcgagtggttttcgccaagaacagtcagttgaagaggaaatgggacgagctgctcgacaagatcatcgacgaccatgtcagcaaagcatcggcacaggagcaacaccacaagcacgatcagcaagaagatcaagagacagacttcgtcgatgtgctcctcagtcttcaggaggagtacagtctcaccagacagcatatcaaggccatactgatggtaaatctcgtctcatacgtagctagcttattatggtaattaaatgtggtcatattttaagtgtgctgacgcttcagtttgaacccatacacaggacatgtttgtggcaggcacagatacgtcatacatagttcttgagtgcgccatggctgagctcatgcgaaagccgaacctcatggccaaacttcaagctgaggtgagggaaaagacacccaagggccaacaaatggtgaccgaggacgacttggccagcatggcctacctaaaggccaccgtgaaggaaacgctccggctacacccaccgctgccgctcctcctcccgcacctctccatgaccgaatgcgacatcgacggctataaagtccccgccagaacccgtgtcatcgtaaacgcttgggctcttggtagagaccctggatcgtgggaggctgccgacaagttcatgccggagaggtttgtggacgtcgtgtcccccgacttcaaagggagggattttcagtttctgccgtttggagctggccgaaggatatgtcccgggataaattttgggatggcgtctgtggagatcatgcttgccaaccttgtctattgttatgattgggagctcccggacggcatgcggcaagaggacctggatatgactgatgtgtttggcatgacgatgcgtcggaaggagaagttatttcttgtcccgagaacacgagatgttaatcatgcataatatctttcatgaattatgtgcacttgtaaagctagatattacactagtatatatggttttcccagttttcaagagggtatgtgggaaacactccaggtactcacattctgccacacaaaaactaccaaccgtcatcccatttctagtccacggcgatcaaatgggttttattgatggtagaaatatcgtggagcacgttatgtttgttgcctacctcatcaagtcttgccatggtaggaaggagcaacccatggtcattaagcttgactttcaaaaaacattcgactcagtttcttggacctcacttatatccactctaagactttgtggtttccaaccattttttggtagaaaccatcctttctacaggcagaacgatatgagacaaggcaagcccctttcaccttatctcttcattattgttgttgatattcttcaacaactaataaataaaaattatagtcacaattctctctcctatccatttacaactacctaccaccaacgacaatagaatacatgggacgacgcccttatcatagttaagttctcaccctaagaccttgaaaccctaaaacacatcttagacgacttcgcttgaaccctgaattgatctgacgtgcttggcatcagatctcatcatcgcaaacagatgatgagaaaccctaacctcagcgcccaaggagacgacaggaatttacgttggcactctgttggttccgtccagaaggacacactcgaggaggatcggagctcagaagacctactcaaagaagaggtgctgtcatccgcttgcacaccgtcctgcgaggactaaaaaccctaacctaaactactagtcggagtcgaggcatcgaaattctcc

SEQ ID NO: 4 - DNA, 3000 bp, Triticum aestivum
  source 1..3000: mol_type = genomic DNA
ctatatcacttggcttagacttggttaagtctcagttgactgagatctagctacatccttatattaaagatccaacggctgctctactttctccttccacgaaattaacttacccaaattgtaaatttagtcaacttacatgtaactattgcagaaggaaggaaaaacatatttcccatgcattggcaggtggataagatacgtacatatgtgatcatggttgcgccgcgcatgtccatcgatggagaaattcaagtccaccaccactaaacgatgaacagaagtggagaaggacacgcaccaaactccaaagtccaaacctcattgtcacgtagcaaatcgcgagcatgggctacgcatccagtcgtggtcagaagatcacagtgatcactcttgtcgaccagctacaaatacgacaccaagggagggtgctacaagcaggccatggcggctcaaacagtgctaccactgctcttatctccccaagcactattgctctatctcttgctcatccctctggtgatcctcctccgggcaacaagcacgagaccggccggcgagcgagccgcagcggacaaccatgggggccgtcccctcccttcgcctccgaacaagctccctctcatcggccacctgcacctggtcggccccgacccgcacgtctccctcgccatcctcgccgccaagcacggcgacggcggcctcatgctcctccgcctcggccagacgcgcgccctcgtcgtctcctccccgcgcgccgccgaggcggtcctgcgcacgcaggacctacgtcttcgcctcgcggcctccgaacgcgctcgtcgacgccctcctggacggcggcgccgacgtcgccttcgccccctacggcgagttctggcggcaggccaggaggctggtcaccacgcacctgctcagcgccaggaagctgcactcgctccgccgcggccgcgagggggaggcgcgcctggtgatggccaagatccagggcgcggcggccgccggcgcccccgtggacatgacgaggctgctcggcagcttcaccaacgacatagcgtgccgcgccgtgtccgggaagttcttccgggaggaaggccggaacgagctgttcagggaggcgatcgacgggaacgtggccgcgtttggcgggttcagcctgctggactacttcccgggcctggccaaggtgggcgtgctcacgcgagtggttttcgccaagaacagtcagttgaagaggaaatgggacgagctgctcgacaagatcatcgacgaccatgtcagcaaagcatcggcacaggagcaacaccacaagcacgatcagcaagaagatcaagagacagacttcgtcgatgtgctcctcagtcttcaggaggagtacagtctcaccagacagcatatcaaggccatactgatggtaaatctcgtctcatacgtagctagcttattatggtaattaaatgtggtcatattttaagtgtgctgacgcttcagtttgaacccatacacaggacatgtttgtggcaggcacagatacgtcatacatagttcttgagtgcgccatggctgagctcatgcgaaagccgaacctcatggccaaacttcaagctgaggtgagggaaaagacacccaagggccaacaaatggtgaccgaggacgacttggccagcatggcctacctaaaggccaccgtgaaggaaacgctccggctacacccaccgctgccgctcctcctcccgcacctctccatgaccgaatgcgacatcgacggctataaagtccccgccagaacccgtgtcatcgtaaacgcttgggctcttggtagagaccctggatcgtgggaggctgccgacaagttcatgccggagaggtttgtggacgtcgtgtcccccgacttcaaagggagggattttcagtttctgccgtttggagctggccgaaggatatgtcccgggataaattttgggatggcgtctgtggagatcatgcttgccaaccttgtctattgttatgattgggagctcccggacggcatgcggcaagaggacctggatatgactgatgtgtttggcatgacgatgcgtcggaaggataagttatttcttgtcccgagaacacgagatgttaatcatgcataatatctttcatgaattatgtgcacttgtaaagctagatattacactagtatatatggttttcccagttttcaagagggtatgtgggaaacactccaggtactcacattctgccacacaaaaactaccaaccttcatcccatttctagtccacgacgatcaaatgggttttattgatggtagaaatatcgtggagcacgttatgtttgttgcctacctcatcaagtcttgccatggtaggaaggagcaacccatggtcattaagcttgactttcaaaaaacattcgactcagtttcttggacctcacttatatccactctaagactttgtggtttccaaccattttttggtagaaaccatcctttctaccggcagaacgatatgagacaaggcaagcccctttcaccttatctcttcattattgttgttgatattcttcaacaactaataaataaaaattatagtcacaattctctctcctatccatttacaactacctaccaccaacgacaatagaatacatgggacgacgcccttatcatagttaagttctcaccctaagaccttgaaaccctaaaacacatcttagacgacttcgcttgaaccctgaattgatctgacgtgcttggcatcagatctcaccatcgcaaacagatgatgagaaaccctaacctcagcgcccaaggagacgacaggaatttacgttggcactctgttggttccgtccagacggacacactcgaggaggatcggagctcagaagacctactcaaagaagaggtgctgtcatccgcctgcacaccgtcctgcgaggactaaaaaccctaacctaaactactagtcggggtcgacacaccgaaattctcc

SEQ ID NO: 5 - protein, 337 aa, Triticum aestivum
MAAQTVLPLLLSPQALLLYLLLIPLVILLRATSTRPAGERAAADNHGGRPLPSPPNKLPLIGHLHLVGPDPHVSLAILAAKHGDGGLMLLRLGQTRALVVSSPRAAEAVLRTQDLRLRLAASERARRRPPGRRRRRRLRPLRRVLAAGQEAGHHAPAQRQEAALAPPRPRGGGAPGDGQDPGRGGRRRPRGHDEAARQLHQRHSVPRRVREVLPGGRPERAVQGGDRRERGRVWRVQPAGLLPGPGQGGRAHASGFRQEQSVEEEMGRAARQDHRRPCQQSIGTGATPQARSARRSRDRLRRCAPQSSGGVQSHQTAYQGHTDGHVCGRHRYVIHSS

SEQ ID NO: 6 - protein, 533 aa, Hordeum vulgare
MAAQPVLPLLLSTQALLLYLLLIPLLILLRATSRRSAGERAAVDNHGGRPLPSPPNKLPLIGHLHMVGSDPHVSLAALAAKHGDGGLMLLRLGQTRALVVSSPRAAEAVLRTQDHVFASRPTNAVVDALLDGGADIAFVPYGEFWRQARRLVTTHLLSARKVHSLRRGREEEARLVMAKIQGAAAAGATVDMTRLLGAFTNDIVCRAVSGKFFREEGRNELFREVIDGNVAAFGGFNLLDYYPGLAKVSMLRRLVFAKTNRLKRKWDDLLDKIIVDHVSQKASPREQHRDRDQQEDEEETDFVDVLLGLQEEYNLTTEHIKAILMDMFVAGTDTSYIVLECAMAELMRKPNLMTKLQAEVGEKTPKGQQMVTEDDLGSMAYLKAVVKETLRLHTPVPLLLPHLSMAECNIDGYTVPAETRVVVNAWALGRDHGSWEAAGEFMPERFGDIVSPDFKGRDFQFLPFGAGRRMCPGINFAMATVEIMLANLVYCYDWELPGGMRQEDLDMTDVFGMTMRRKEKLFLVPISRNVNRA

SEQ ID NO: 7 - DNA, 1602 bp, Hordeum vulgare
  source 1..1602: mol_type = other DNA
atggcggctcaacctgtgctgccactgctcttatctacccaagcactgttgctctatctcttgctcatccctctgctgatcctcctccgggcaacgagcaggagatcggccggcgagcgagctgcagtggacaaccatgggggccgtcccctcccttcgcctcccaacaagctccctctcatcggccacctgcacatggtcggctccgacccccacgtctccctcgccgccctcgccgctaagcacggcgacggcggtctcatgctcctccgcctcggccagacgcgcgccctcgtcgtctcctccccgcgcgccgccgaggcggtcctgcgcacgcaggaccacgtcttcgcctcgcggccgacgaacgcggtcgtcgacgccctcctcgacggcggcgctgacatcgccttcgtcccctacggcgagttctggcggcaggcgaggaggctggtcaccacgcacctgctcagcgccaggaaggtgcactccctccgccgcggccgcgaggaggaagcgcgcctggtgatggccaagatccagggcgcggcggccgccggcgccaccgtggacatgacgaggctgctcggcgccttcaccaacgacatagtgtgccgcgccgtgtccgggaagttcttccgggaggaaggccggaacgagctgttcagggaggtcatcgacgggaacgtggccgcgtttggcgggttcaacctgctggactactacccgggcctggccaaggtgagcatgctcaggcgactggtgtttgccaagaccaaccggttgaagaggaaatgggacgacctgctcgataagatcatcgtcgatcatgtcagccaaaaagcatcgccacgggagcagcaccgcgaccgcgatcagcaagaagatgaagaagagacagacttcgtcgatgtgctcctcggtcttcaggaggagtacaatctcaccacagagcatataaaggccatattgatggacatgtttgtggcaggcacagatacttcatacatagttctcgagtgcgccatggctgagctcatgcgaaagccgaacctgatgaccaaacttcaagctgaggtgggggagaagacacccaagggccaacaaatggtgaccgaggacgacttgggcagcatggcctacctgaaggccgtcgtgaaggagacgctccggctacacacaccggtgccgctcctcctcccgcacctctccatggccgaatgcaacatcgacggttatacagttcccgctgaaacccgtgtcgtcgtaaacgcttgggctcttggtagagaccatggatcgtgggaggctgccggcgagttcatgccggagaggtttggcgacatcgtgtcccccgacttcaaagggagggatttccagtttcttccgtttggagctggacgaaggatgtgccccgggataaatttcgcgatggctactgtggagatcatgctcgctaaccttgtctattgttatgattgggagctcccgggtggaatgcggcaagaggacctcgacatgacagatgtgtttggcatgacgatgcgccggaaggagaagttgtttcttgtcccgatatcgaggaatgttaatcgtgcataa

SEQ ID NO: 8 - DNA, 2942 bp, Hordeum vulgare
  source 1..2942: mol_type = genomic DNA
cttcgggaattttgttctacttcaaataatttggtgcttcacaaaaatttcgaaaatttaagaaagtgggaattttgaaatagaatgtttaataaattataaaatgtttgtggattcaaaaatacccgcgattttgcagaaaatgttagaaattttgaaaacaaatatttgagaaatcaaacaatgttcatgattttttaaaagttcatgaagtactttttataatgaaattgtgcaaaattttgtcaattctaaaaatgatcatgaatggaaaaatattctaaaagttcaaaaaaacaatgatttgtgacttataaaatagtttttcatttataaaatgtttgctgatttagaaaattatcatgcatttttttgtcccgttgcaacgcacgggcccttttgttagtaagtatacaaaagttttagttggttttaaattttgtgaaaacaaaatgtggcaaggtggcacaaacacagggtgtgacattttccttaaaaaaaacctttcttcttggtataatcttctttcttctcccatcgtttctccttccacaaaatcgagctatccagattgtaaatttagtcaacttacgtatggctatagcgcaaaaaaaaaaaacatattttccatgcatttgcaggtggataagatacgtacgtatgtgatcatggttccgccgcgcctatccatcgatcgacaaattcaagtcccactacgtactaaacgttgaacagaagaggagaaggacacactccaaactccaaagactccaaacctcattgtgaggtagcaaatcgggccatgtgctacacatccatccgtggtccgtactcgatcactcttctagtactcgaccagctacaaatactgacaccaagggagggtgcatgtgccgtactgctagcaagcaggcatggcggctcaacctgtgctgccactgctcttatctacccaagcactgttgctctatctcttgctcatccctctgctgatcctcctccgggcaacgagcaggagatcggccggcgagcgagctgcagtggacaaccatgggggccgtcccctcccttcgcctcccaacaagctccctctcatcggccacctgcacatggtcggctccgacccccacgtctccctcgccgccctcgccgctaagcacggcgacggcggtctcatgctcctccgcctcggccagacgcgcgccctcgtcgtctcctccccgcgcgccgccgaggcggtcctgcgcacgcaggaccacgtcttcgcctcgcggccgacgaacgcggtcgtcgacgccctcctcgacggcggcgctgacatcgccttcgtcccctacggcgagttctggcggcaggcgaggaggctggtcaccacgcacctgctcagcgccaggaaggtgcactccctccgccgcggccgcgaggaggaagcgcgcctggtgatggccaagatccagggcgcggcggccgccggcgccaccgtggacatgacgaggctgctcggcgccttcaccaacgacatagtgtgccgcgccgtgtccgggaagttcttccgggaggaaggccggaacgagctgttcagggaggtcatcgacgggaacgtggccgcgtttggcgggttcaacctgctggactactacccgggcctggccaaggtgagcatgctcaggcgactggtgtttgccaagaccaaccggttgaagaggaaatgggacgacctgctcgataagatcatcgtcgatcatgtcagccaaaaagcatcgccacgggagcagcaccgcgaccgcgatcagcaagaagatgaagaagagacagacttcgtcgatgtgctcctcggtcttcaggaggagtacaatctcaccacagagcatataaaggccatattgatggtaattaaatcctctcatgccgtcatactcctacgtgcgtagctggctgatttaagtgtgctgacgcttcaggttgaactgaatccgtacgcaggacatgtttgtggcaggcacagatacttcatacatagttctcgagtgcgccatggctgagctcatgcgaaagccgaacctcatgaccaaacttcaagctgaggtgggggagaagacacccaagggccaacaaatggtgaccgaggacgacttgggcagcatggcctacctgaaggccgtcgtgaaggagacgctccggctacacacaccggtgccgctcctcctcccgcacctctccatggccgaatgcaacatcgacggttatacagttcccgctgaaacccgtgtcgtcgtaaacgcttgggctcttggtagagaccatggatcgtgggaggctgccggcgagttcatgccggagaggtttggcgacatcgtgtcccccgacttcaaagggagggatttccagtttcttccgtttggagctggacgaaggatgtgccccgggataaatttcgcgatggctactgtggagatcatgctcgctaaccttgtctattgttatgattgggagcttccgggtggaatgcggcaagaggacctcgatatgacagatgtgtttggcatgacgatgcgccggaaggagaagttgtttcttgtcccgatatcgaggaatgttaatcgtgcataatatttggcacaaattttgtgcatggtaaggctagatggtgtatttgtatgtatggttttccagctttatcgaaaaatactttcgccccgttttatagatgaagcaaaccaccgaaccacaacatccaacaacagtcacaataacacatacacacgccgcactagaggtagcacaacaacacaaggtacgaaggtaacgttgagggcacaacacaacaagcccaaacaaaggaaaacaacaaggcggcgctgcaaaacaaaaatgatcctctaatccggcttcggaggtggaggagggagcggccgcgccaagcggagagccattgcaagaag

SEQ ID NO: 9 - DNA, 20 bp, synthetic construct
  source 1..20: mol_type = other DNA
ccgggcaacaagcacgagac

SEQ ID NO: 10 - DNA, 20 bp, synthetic construct
  source 1..20: mol_type = other DNA
agggcgtcgacgagcgcgtt

SEQ ID NO: 11 - DNA, 21 bp, synthetic construct
  source 1..21: mol_type = other DNA
gtcgtggtcagaagatcacag

SEQ ID NO: 12 - DNA, 20 bp, synthetic construct
  source 1..20: mol_type = other DNA
gatgagagggagcttgttcg

SEQ ID NO: 13 - DNA, 18 bp, synthetic construct
  source 1..18: mol_type = other DNA
ctcatgctcctccgcctc

SEQ ID NO: 14 - DNA, 18 bp, synthetic construct
  source 1..18: mol_type = other DNA
cgccagaactcgccgtag